European Patent Application EP 4 721 754 A1, published April 8, 2026. Title: 一种口服递送的多肽衍生物. Applicant: 杭州先为达生物科技股份有限公司. Application CN. The sequence listing filed with the application follows.

SEQUENCE LISTING (5 sequences)

SEQ ID NO: 1 - protein, 37 aa, synthetic construct
KCNTATCATQRLAEFLRHSSNNFGPILPPTNVGSNTP

SEQ ID NO: 2 - protein, 36 aa, synthetic construct
  MOD_RES 36: note = trans-Hyp
KCNTATCATQRLADFLRHSSNNLKPILPPTNVGSNT

SEQ ID NO: 3 - protein, 32 aa, synthetic construct
ASQLSTAVLGRLSQELHRLQDYPRTDVGSGSP

SEQ ID NO: 4 - protein, 32 aa, synthetic construct
ASQLSTAVLGRLSDELHRLQDYPRTDVGSGSP

SEQ ID NO: 5 - protein, 32 aa, synthetic construct
CSNLSTCVLGKLSQELHKLQTYPRTNTGSGTP